European Patent Specification EP 3 307 070 B1, published October 29, 2025. Title: Growth and Survival Compositions for Cells Capable of Producing Antibodies and Methods Related Thereto. Applicant: Emory University. The sequence listing filed with the application follows.

SEQUENCE LISTING (13 sequences)

SEQ ID NO: 1 - protein, 250 aa, Homo sapiens [sequence omitted]

SEQ ID NO: 2 - protein, 212 aa, Homo sapiens
MNSFSTSAFGPVAFSLGLLLVLPAAFPAPVPPGEDSKDVAAPHRQPLTSSERIDKQIRYILDGISALRKETCNKSNMCESSKEALAENNLNLPKMAEKDGCFQSGFNEETCLVKIITGLLEFEVYLEYLQNRFESSEEQARAVQMSTKVLIQFLQKKAKNLDAITTPDPTTNASLLTKLQAQNQWLQDMTTHLILRSFKEFLQSSLRALRQM

SEQ ID NO: 3 - protein, 135 aa, Homo sapiens
CESSKEALAENNLNLPKMAEKDGCFQSGFNEETCLVKIITGLLEFEVYLEYLQNRFESSEEQARAVQMSTKVLIQFLQKKAKNLDAITTPDPTTNASLLTKLQAQNQWLQDMTTHLILRSFKEFLQSSLRALRQM

SEQ ID NO: 4 - protein, 250 aa, Pan troglodytes [sequence omitted]

SEQ ID NO: 5 - protein, 250 aa, Canis lupus
MPASSPSLLAPKGPPGDMGGPVREPALSVALWLSWGAALGAVACAMALLTQQTELQNLRREVARLQRTGGPSEKEEGYPWLSLQEQSPDALEAWENGERSRRKRAALIHKQKKKHSVLHLVPINITSKEDSDVTEVMWQPALKRGRGLEAQGYVVRVWDSGIYLLYSQVLFHDVTFTMGQVVSREGQGRQETLFRCIRSMPSNPDWAYNSCYSAGVFHLHQGDILSVTIPRGRAKLSLSPHGTFLGFVKL

SEQ ID NO: 6 - protein, 250 aa, Bos taurus
MPASSPSLLSPKGPQGDMGGPVREPALSVALWLSWGAALGAVACAMVLLTQQTELQTLRREVTRLQRNGGPSEKGEGNPWLNLQEQSPDGTEGQENGERSRRRRAVLTRKHKKKRSVLHLVPINITSKEDSDVTEVMWQPALQRGRGLEAQGYVVRVWDAGVYLLYSQVLFHDETFTMGQMVSREGQGRQETLFRCIQSMPSNPDWAYNSCYSAGVFHLHQGDILSVVIPRARAKLSLSPHGTFLGLVKL

SEQ ID NO: 7 - protein, 241 aa, Mus musculus
MPASSPGHMGGSVREPALSVALWLSWGAVLGAVTCAVALLIQQTELQSLRREVSRLQRSGGPSQKQGERPWQSLWEQSPDVLEAWKDGAKSRRRRAVLTQKHKKKHSVLHLVPVNITSKADSDVTEVMWQPVLRRGRGLEAQGDIVRVWDTGIYLLYSQVLFHDVTFTMGQVVSREGQGRRETLFRCIRSMPSDPDRAYNSCYSAGVFHLHQGDIITVKIPRANAKLSLSPHGTFLGFVKL

SEQ ID NO: 8 - protein, 240 aa, Rattus norvegicus
MPASSPGNMGGSVREPALSVTLWLSWGAVLGAVTCAVALLIQQAELQSLRREVSRLQRSGGASQKRGEPPWQSLWEQSPDVLGAWKDGAKSRRRRAVLTQKHKKKQSVLHLVPINITSKDSDMTEVMWQPALRRGRGLEAQGDTVRVRDTGIYLLYSQVLFHDVTFTMGQVVSREGQGRRETLFRCIKSMPSDPDRAYNSCYSAGVFHLHQGDIITVKIPRANAKLSLSPHGTFLGFVKL

SEQ ID NO: 9 - protein, 212 aa, Pan troglodytes
MNSVSTSAFGPVAFSLGLLLVLPAAFPAPVPPGEDSKDVAAPHRQPLTSSERIDKQIRYILDGISALRKETCNKSNMCESSKEALAENNLNLPKMAEKDGCFQSGFNEETCLVKIITGLLEFEVYLEYLQNRFESSEEQARAVQMSTKVLIQFLQKKAKNLDAITTPDPTTNASLLTKLQAQNQWLQDMTTHLILRSFKEFLQSSLRALRQM

SEQ ID NO: 10 - protein, 212 aa, Macaca mulatta
MNSFSTSAFGPVAFSLGLLLVLPAAFPAPVLPGEDSKNVAAPHSQPLTSSERIDKHIRYILDGISALRKETCNRSNMCESSKEALAENNLNLPKMAEKDGCFQSGFNEDTCLVKIITGLLEFEVYLEYLQNRFESSEEQARAVQMSTKVLIQFLQKKAKNLDAITTPEPTTNASLLTKLQAQNQWLQDMTTHLILRSFKEFLQSNLRALRQM

SEQ ID NO: 11 - protein, 207 aa, Canis lupus
MNSLSTSAFSLGLLLVMATAFPTPGPLAGDSKDDATSNSLPLTSANKVEELIKYILGKISALRKEMCDKFNKCEDSKEALAENNLHLPKLEGKDGCFQSGFNQETCLTRITTGLVEFQLHLNILQNNYEGDKENVKSVHMSTKILVQMLKSKVKNQDEVTTPDPTTDASLQAILQSQDECVKHTTIHLILRSLEDFLQFSLRAVRIM

SEQ ID NO: 12 - protein, 211 aa, Mus musculus
MKFLSARDFHPVAFLGLMLVTTTAFPTSQVRRGDFTEDTTPNRPVYTTSQVGGLITHVLWEIVEMRKELCNGNSDCMNNDDALAENNLKLPEIQRNDGCYQTGYNQEICLLKISSGLLEYHSYLEYMKNNLKDNKKDKARVLQRDTETLIHIFNQEVKDLHKIVLPTPISNALLTDKLESQKEWLRTKTIQFILKSLEEFLKVTLRSTRQT

SEQ ID NO: 13 - protein, 211 aa, Rattus norvegicus
MKFLSARDFQPVAFLGLMLLTATAFPTSQVRRGDFTEDTTHNRPVYTTSQVGGLITYVLREILEMRKELCNGNSDCMNSDDALSENNLKLPEIQRNDGCFQTGYNQEICLLKICSGLLEFRFYLEFVKNNLQDNKKDKARVIQSNTETLVHIFKQEIKDSYKIVLPTPTSNALLMEKLESQKEWLRTKTIQLILKALEEFLKVTMRSTRQT